European Patent Application EP 4 796 638 A1, published August 26, 2026. Title: A transformed plant with modified flower color and a new compound contained therein. Applicant: Suntory Holdings Limited. The sequence listing filed with the application follows.

SEQUENCE LISTING (12 sequences)

SEQ ID NO: 1 - DNA, 1257 bp, synthetic construct
  source 1..1257: mol_type = other DNA
atgaagcacagttcggatatctgcatagttggggccggtatatcaggacttacatgtgcctcgcatctcttggacagtccagcatgtaggggtctttctctccgcatctttgacatgcaacaagaagccggaggccgaattaggtccaagatgcttgacggaaaagcctcgattgagttgggtgctggtaggtatagccctcagttgcatcctcacttccaatctgccatgcagcactacagtcagaagagtgaggtctacccgtttacgcaactcaagttcaagagccacgttcaacagaagctcaaacgcgctatgaacgagttgagtcccagattgaaggagcatgggaaagagtccttcttgcagttcgtgtcccgataccaagggcatgatagcgcagtaggcatgattcgctcaatgggctatgatgccctttttcttcccgacatttccgccgagatggcatatgacatagtgggcaaacaccccgaaatccagtctgttaccgacaatgacgcaaaccagtggtttgcagcagagactggctttgcaggactgattcaggggattaaggcaaaggttaaggctgctggagcccgtttctcgctgggttatcggcttctttcagttcgcacagatggggatggctacttgttacaattagcaggtgatgatggttggaaactcgagcacagaactaggcacttgatactcgccattccaccgtctgctatggctggcctgaatgtcgactttcctgaggcttggtctggggctagatacgggagcttgcctctcttcaagggatttctgacctacggtgaaccatggtggctcgactacaaacttgacgatcaagtcttgatcgtggacaatccgcttaggaagatctacttcaagggggataagtacctcttcttctacaccgactccgaaatggccaactactggagaggttgcgtagctgagggtgaggacgggtacttggaacagatccgtacacatctcgcttctgcgctagggatcgtgcgtgagcgtattcctcaaccgttagctcacgtgcacaaatactgggcacatggtgtcgagttttgtcgggattctgacattgaccacccttctgccctctcacatcgggattcaggaattatcgcctgtagcgatgcatacactgagcattgtggttggatggaaggagggttactaagtgctcgggaagcttcacgtttgctactgcaacgaattgcagcctaa

SEQ ID NO: 2 - protein, 418 aa, Chromobacterium violaceum
MKHSSDICIVGAGISGLTCASHLLDSPACRGLSLRIFDMQQEAGGRIRSKMLDGKASIELGAGRYSPQLHPHFQSAMQHYSQKSEVYPFTQLKFKSHVQQKLKRAMNELSPRLKEHGKESFLQFVSRYQGHDSAVGMIRSMGYDALFLPDISAEMAYDIVGKHPEIQSVTDNDANQWFAAETGFAGLIQGIKAKVKAAGARFSLGYRLLSVRTDGDGYLLQLAGDDGWKLEHRTRHLILAIPPSAMAGLNVDFPEAWSGARYGSLPLFKGFLTYGEPWWLDYKLDDQVLIVDNPLRKIYFKGDKYLFFYTDSEMANYWRGCVAEGEDGYLEQIRTHLASALGIVRERIPQPLAHVHKYWAHGVEFCRDSDIDHPSALSHRDSGIIACSDAYTEHCGWMEGGLLSAREASRLLLQRIAA

SEQ ID NO: 3 - DNA, 2997 bp, synthetic construct
  source 1..2997: mol_type = other DNA
atgtcgatcttggactttcctcgtatccacttcaggggttgggctcgggtcaatgctccgactgccaatcgcgatccgcatggacacattgatatggcgtctaatacagttgcaatggcaggggagccgtttgatttggccagacatccaactgagtttcacagacatttgcgttctcttggtccccgctttggcctcgatggccgagccgatcccgaaggaccgtttagtctggcagaaggctacaacgctgccggtaacaaccacttctcttgggagagtgccacggtgtctcacgttcagtgggacgggggtgaggcagaccgcggagatggactggtcggtgctagactcgctctttggggtcattacaatgattaccttcgcacaacgtttaatcgggctaggtgggtggatagcgatccaaccagaagagacgctgcacagatctatgctggccaattcaccatctcgcctgcaggtgctggacctggaacgccgtggctcttcacagctgacatcgacgacagtcatggtgctcgatggaccagaggtgggcatattgccgagcgtggtggacatttcttggacgaggagtttggcttggctcgcttgtttcaattctccgtgccaaaggaccatcctcacttcttgtttcaccctggtccctttgactcagaagcctggcggaggctccagcttgctctcgaggatgacgacgttctcgggttgactgttcagtacgcattgttcaacatgtctactcctccgcaacccaattccccggttttccatgatatggtgggggtagtcggactttggcgtaggggcgaacttgccagttatcctgcagggcggttacttcggcctaggcaacccggtttgggtgacttgaccttgcgtgtgaatggcggtagagtcgctctgaaccttgcctgtgcaattccattctctactcgagccgctcagccgtcggcaccggaccgcctcacaccggacttaggggcaaagctgcctcttggggacttacttctcagggacgaggatggtgccttgctggcaagggtcccacaggccctttaccaggactactggacgaatcatgggatagttgacttgcctttgcttagagaaccacgcggctctctaaccttaagtagcgagctagccgaatggcgggagcaggattgggtcactcagtcagatgccagtaacctttacctcgaggctcctgatcgaagacacggaagattttttcccgagtcgattgcccttcgctcatacttccgtggggaggcaagagccagacctgacattccccaccgtatcgaaggcatgggcctcgttggtgtggaatcacgtcaagacggggatgccgcagagtggcggttgacagggttaaggcctggtcctgctcgtatcgtgctagatgatggggccgaggccatacccctgagggtactcccggacgattgggcattagacgatgccacagtcgaggaggtagactacgcttttttgtaccgtcatgttatggcgtattacgaactcgtgtacccgttcatgagcgacaaagtgttcagcctagccgacaggtgcaagtgcgaaacttacgcccgccttatgtggcagatgtgtgatccgcaaaaccgcaacaagtcctactacatgccctctacccgagagttgtctgctccgaaagctcgactgttcctcaagtacctcgctcacgtggagggccaagctagactccaagcacctccacccgcaggaccggctcggatagagagtaaggcacaactcgcagctgaacttagaaaggctgtggatttggaattaagcgtgatgcttcagtacttgtatgccgcttactccattcccaactatgcacagggtcagcaacgtgtcagggacggggcttggaccgccgagcaactgcaacttgcttgtgggtctggtgatagacgacgtgacggaggtatcagggccgctttactagagatagcccacgaggagatgatccactacttggtcgttaacaacttgttgatggcccttggcgaacccttttacgccggagtaccgttgatgggcgaagcagcacgtcaagcattcggattggatacagagttcgcgttagagcctttcagtgagtcaactctcgcacgtttcgtccgacttgaatggcctcacttcattcctgctccggggaagtcaattgctgactgctacgccgctattcggcaagcctttctggatttaccggacctctttggtggagaagctggtaaacgcggcggagagcaccacctatttctcaatgagctgacaaaccgtgcacatcctgggtatcagttggaggtgtttgacagggactccgctctcttcggtattgcctttgttaccgatcaaggggaagggggtgccttagactcacctcactatgagcattcccatttccagaggctccgtgagatgtccgcacgcatcatggcccaatctgctccattcgaacctgccctacctgcactccgtaaccccgttttggatgagtcaccagggtgtcaaagggttgccgacggaagagccagggcactcatggctctgtaccaaggcgtttatgagcttatgttcgcaatgatggcccaacactttgcagtgaaaccactcggtagtcttcgaaggtcacgtcttatgaatgcagccattgacctcatgactgggcttttgcggcctctcagctgtgcattgatgaatttgccttctgggattgcaggacgaactgccggtccaccattgccgggcccagttgacacccgttcgtacgatgactacgccttggggtgtcgtatgctcgctcgccgctgcgagcggctcctggaacaggcaagcatgttggagcctgggtggctgccagatgcacagatggagctgctggatttctaccgaaggcagatgctcgatctagcttgtggaaagttatcccgggaggcctaa

SEQ ID NO: 4 - protein, 998 aa, Chromobacterium violaceum
MSILDFPRIHFRGWARVNAPTANRDPHGHIDMASNTVAMAGEPFDLARHPTEFHRHLRSLGPRFGLDGRADPEGPFSLAEGYNAAGNNHFSWESATVSHVQWDGGEADRGDGLVGARLALWGHYNDYLRTTFNRARWVDSDPTRRDAAQIYAGQFTISPAGAGPGTPWLFTADIDDSHGARWTRGGHIAERGGHFLDEEFGLARLFQFSVPKDHPHFLFHPGPFDSEAWRRLQLALEDDDVLGLTVQYALFNMSTPPQPNSPVFHDMVGVVGLWRRGELASYPAGRLLRPRQPGLGDLTLRVNGGRVALNLACAIPFSTRAAQPSAPDRLTPDLGAKLPLGDLLLRDEDGALLARVPQALYQDYWTNHGIVDLPLLREPRGSLTLSSELAEWREQDWVTQSDASNLYLEAPDRRHGRFFPESIALRSYFRGEARARPDIPHRIEGMGLVGVESRQDGDAAEWRLTGLRPGPARIVLDDGAEAIPLRVLPDDWALDDATVEEVDYAFLYRHVMAYYELVYPFMSDKVFSLADRCKCETYARLMWQMCDPQNRNKSYYMPSTRELSAPKARLFLKYLAHVEGQARLQAPPPAGPARIESKAQLAAELRKAVDLELSVMLQYLYAAYSIPNYAQGQQRVRDGAWTAEQLQLACGSGDRRRDGGIRAALLEIAHEEMIHYLVVNNLLMALGEPFYAGVPLMGEAARQAFGLDTEFALEPFSESTLARFVRLEWPHFIPAPGKSIADCYAAIRQAFLDLPDLFGGEAGKRGGEHHLFLNELTNRAHPGYQLEVFDRDSALFGIAFVTDQGEGGALDSPHYEHSHFQRLREMSARIMAQSAPFEPALPALRNPVLDESPGCQRVADGRARALMALYQGVYELMFAMMAQHFAVKPLGSLRRSRLMNAAIDLMTGLLRPLSCALMNLPSGIAGRTAGPPLPGPVDTRSYDDYALGCRMLARRCERLLEQASMLEPGWLPDAQMELLDFYRRQMLDLACGKLSREA

SEQ ID NO: 5 - DNA, 1290 bp, synthetic construct
  source 1..1290: mol_type = other DNA
atgaagcgtgcaatcattgtgggaggaggacttgcagggggcttgacagctatctatctagccaaacgcggttatgaggtccatgtggttgagaaacgtggtgaccctctacgtgacttgagcagttacgtggatgtcgtttcttctagagctatcggtgtgtccatgacagttcgtgggatcaaatcagtcctcgctgctgggattcctcgtgctgaactcgatgcatgtggtgaaccgatagtcgctatggcattcagtgtgggagggcagtatcggatgagggagttgaagcccttagaggactttcgcccactgagcttgaatcgagctgcctttcaaaagctgttgaacaagtacgccaacttagctggagtacgctactacttcgagcacaaatgcctcgatgtggatcttgatggaaagtccgttctcattcagggcaaagatgggcaacctcaaaggctgcaaggtgacatgatcatcggtgccgatggtgcacactctgccgttcgccaggctatgcaatccggcttgagacgtttcgagttccaacagaccttctttcgccatgggtacaagaccttggttcttccagacgctcaagcactaggttacaggaaggatacgctgtactttttcggcatggatagtgggggactttttgccggtagagctgcaaccataccggatgggtccgtaagcattgccgtttgtctcccatactcgggctcaccttcactgactactactgacgagcctactatgcgagcctttttcgaccgttactttggcggtttacctagagacgcacgagacgaaatgcttcgtcagttccttgccaaaccgtctaatgacctcattaacgttcggtcttcgactttccactacaagggtaacgtgctcctcttgggagatgcagcacatgccacagcaccctttttggggcaagggatgaatatggccttagaagacgcgagaacgttcgttgagctcttggaccgacatcaaggggatcaggacaaagcctttcccgagtttaccgagttgaggaaggtccaagctgacgcaatgcaagacatggctagggccaactatgacgtgctttcatgttcgaaccccattttcttcatgagggcacggtacacacggtacatgcactctaagtttccgggcttgtatccgcctgatatggccgagaagctctacttcaccagtgaaccatacgatagacttcagcagatacagcggaagcagaatgtgtggtacaagattggtagggtcaattaa

SEQ ID NO: 6 - protein, 429 aa, Chromobacterium violaceum
MKRAIIVGGGLAGGLTAIYLAKRGYEVHVVEKRGDPLRDLSSYVDVVSSRAIGVSMTVRGIKSVLAAGIPRAELDACGEPIVAMAFSVGGQYRMRELKPLEDFRPLSLNRAAFQKLLNKYANLAGVRYYFEHKCLDVDLDGKSVLIQGKDGQPQRLQGDMIIGADGAHSAVRQAMQSGLRRFEFQQTFFRHGYKTLVLPDAQALGYRKDTLYFFGMDSGGLFAGRAATIPDGSVSIAVCLPYSGSPSLTTTDEPTMRAFFDRYFGGLPRDARDEMLRQFLAKPSNDLINVRSSTFHYKGNVLLLGDAAHATAPFLGQGMNMALEDARTFVELLDRHQGDQDKAFPEFTELRKVQADAMQDMARANYDVLSCSNPIFFMRARYTRYMHSKFPGLYPPDMAEKLYFTSEPYDRLQQIQRKQNVWYKIGRVN

SEQ ID NO: 7 - DNA, 576 bp, synthetic construct
  source 1..576: mol_type = other DNA
atggagaatcgcgaaccaccgttgttgccggctagatggtccagtgcatacgtgtcgtactggtcacctatgctacctgacgaccaacttacctctgggtactgttggttcgactacgaacgggacatctgcaggatagacggcctgtttaacccgtggagtgagcgcgatacaggctatcgcctctggatgtccgaggtagggaatgctgcatctggaaggacctggaagcagaaggttgcctatgggagagaacggactgcattgggtgagcagctttgtgagcgtccactggacgatgagacaggtccctttgccgagcttttccttcctcgagacgtcttgcgaagactcggtgctcgtcacattgggcgtagggttgtcttaggtcgtgaagccgatggatggcgctaccaacgtcctggcaaaggtcctagcactctctacctcgatgcagcctctgggactccgttacggatggttacgggagatgaggctagcagggcatcgttgcgagacttcccaaacgtgtcagaagccgagattcccgatgctgtgtttgctgccaagagataa

SEQ ID NO: 8 - protein, 191 aa, Chromobacterium violaceum
MENREPPLLPARWSSAYVSYWSPMLPDDQLTSGYCWFDYERDICRIDGLFNPWSERDTGYRLWMSEVGNAASGRTWKQKVAYGRERTALGEQLCERPLDDETGPFAELFLPRDVLRRLGARHIGRRVVLGREADGWRYQRPGKGPSTLYLDAASGTPLRMVTGDEASRASLRDFPNVSEAEIPDAVFAAKR

SEQ ID NO: 9 - DNA, 1028 bp, Eustoma grandiflorum
  source 1..1028: mol_type = other DNA
caattagttttttttccttcttctttttattcgactcaatactcaattaggtttaatccattgcccatcaaaaagttgtcttgatggataaacttttcagcacttaatactaatccaaaatatcatttaagcatcacatgccgtgacactccagatggttaaaaatgaacgtacttgaactcaattgtaatgatcaattactcttagaagtcaaaataatgtcaattacaacacaacaacaaccagtcttagaggctcccgcctatggcgaagtatagggagggtcggatgtacgtaactagggctgttcaacgaaccaaacagtttacgaactgttcgagtttggttcgtgttcggtttgtatttgttcgttaatggttgataaacgatccgaatttgaacagctatttgggttcgtttactaaaatgagccgaactattcacgaactattcggctcgtttaaacagttaaagggttatcaagccgaattcgaaccaattttaaaattcgtttagctaaaagaaccgagccaaacatttcatttagccaaacgaatccgaattcgaaaacgtagttttcggttctgctctattagttaacagccctatacgtaatcatactcataagttgtgagaaacacacagatgttttttttccgatgacccataatgaaaattgcatcaaactgtgccgatcaactgttactttactatataaaaaacacggtaagtcattttgttttatttcattatattccaaatacaaggaagaatgcgtcaagtaagacttctaaattttgtgtactagtagaagaagtttgttgggtttatagttgttgtgctaatgttagttggagactttcttgattcagaccacgtggttgtccaagatacacaaaggtcatgcaataaaattatatgtccacaaggtctatatataacgtgaaaaattgaaacacagcatagggcttgataatttcattcatcaaaagtaaagatcaaagcacttcatttagcaatcaggaatc

SEQ ID NO: 10 - DNA, 1003 bp, Ipomoea nil
  source 1..1003: mol_type = other DNA
tgtaatttttccatcaataaatgataagggaaaatgtcacttttttcctttaaattgcatggcatgcttatagcactttttttccttaattatttatctatatgattattttgaatgcggtgtttctccatcttctatgttaaatggtcgtttgaattgttaaaatatgattattttgaaagcggtgtttctccctcttctatgttaaatggtcgtttgaattgttaaaaataagggcaaaatatgtatttcaagttattttctttctccaacttatatgtagaaattagaataaatctgaaaaaaataggcaacaaattaatgcacactttggttgttgtttttttttttttttttttttttttttaattctcacatataagcaataatttgttggggaagaaaaatgacttgaaatgcttattttgcgcttatttttaatcgttcaaacgctcatttaattaacatgaggggattgcatgtcactttcaaaataactaagataatgtgaatccatgaataatttaggagaaaaaagtgccataagtataaaatcatagacaaatatgattaataattaataataagaaaaaagtgtcaaattggcccataagtcttctagctcaaaaacgctccaatgaagtactctaaattaaagcagtaaaatagtgcaattagttatattattacccattaagcattgaagtgtcgttagccatgctaacatgtggtgttttaatatttattattattattattgttggaataataatatatagtatataaggttacgttgtgttgttgggtcaccaaacggggggttgatatcgagtatgaagcacgcacgtgcatcgacgagcggaccaaacagtcatgagcttaactaataacgtgtataaaactttgatcattctataaggcttttcacttgcagcagattaattagatccacaatatactttaatttcttggctagaagcttagcttattgatccgaggaaaa

SEQ ID NO: 11 - DNA, 2908 bp, Rosa hybrida
  source 1..2908: mol_type = other DNA
cagcaagagttgaagaaatagggacagagccatccatgtgctttgatgaatctgatgggatacaaaatgtgaaagattcacttgctgatttatccagaatttcttcatatagtgaggagaatgttgaaagatctaatgatgagcactctgttaaactagacggaattcatgtgcagcacgagtgtcatgagggcagtgaagaagacaaacctgatggtaagagcggtgagaatgcagttgatctggctaatcatggcatggctcgaactgatttttgtcagataacagaagagattgagaatggagtagtcatcactgagatgagcaacattgccaaccctgataaaactgatattccaaacggggtgcctcaaaatgagactgatgatggatttaataacactcaggatgatgctaatacaaaggaagtgacagaagagaattctgacagacgtgcgaaggaagtgacagaagagaattctgacaaagatgttttgaagaatatccttgaattctcacgtgcttcttctgtggtggattttgaaattccagtgttggatgtgaaatttacttctcttgaaagttgcagtgccacttgttctcttgcagcccttttgtctgaatcgccggaatcaatgactgaagcaccttgtgtgaggcaaattgatgatgtgcccccggttggtgaggagtctagcttgattttggtggaagatcgggagccggttggtcctactcctgatggtaatttttctgtggatatggattactatagtgtagcagaacctttgagcacatgggatgcgaatctgcagtgtgaaacatcaaatagccatgagacttttgctgcaagtctcatttgatagcttctgtgttaataactttgttagtctgtacataaatttgtctagacaagaattggtcgtgtactatcgtgtgtttttgccgtgctttagtactcatgaaccaattcagagaaaactggctgcatattttgaggagtctctgaattcttcaatgctcaactggtatgcatgtaggtggcatatcacttcagggattcttctattctttaactttacgcatcttgacattttgtatataacaaaatcaggtctattgggtgaaagtaattggctagaatggaaagctctacggttttaccgcaggtcaattttcatagctccacaagtgaattgaaaatgctcataggctttatgtttgtcctccacctctggcgacgatgtttgttggggagttaactcaaacctaccaccaaactcgaacccatcttccataatttataatacaaatttgcgatcatttgttcatccaattattgtgacactcggctaccacccaaaatatcggtcacagacccaaacgtattgtcacaacaaatcgtgtctctcgcattaaacacagctagaaagaagagttgaacccacaattcgagcacccactacctatgtacgaagtcatgagttcgagtcaccataggggtagaagtgaaatcatttgatcatctttaaagaaataaaaggaagagttgaacccacaattggctcttgtcccaaaaagaactaatagttcagtgcaccgacgtgtatttgcaccgacataaatggattgttagattatattaaatacactcttaggttattaataaaaatattaattataaatatcaaaagttgagatcatcttataaatgttgggtcagttacaccgtcggtgcatagaataatttccaaactatataatagccttcattttctgatttagctcatgggacatgattgctataaataattgtactcgtagaggcatacttgtgtctttttatacagttgtactgaagctcagaaaagtttatgaaggtgagaactgagaagggcaaggcatttggtagttgaggtatatgagagcatgaaccccatgcattgcagctaccacctctcttttttccttcttcccatacaaataaaaccaactcttctcacctaagtctatcatctttatttatggcagctcttgcttaattagctcatctatattatattatttatctataatatgtgtcactctgttacctaccagcccaaaataaaactgataatagtcaatttgatgatattttttgttttttgttttgttttgtcttttttgtattgatttttttaaaattaaaatgacttcattttttgtttttgtttttttttctatttttttttatagaaaaattggcaaactttcattatctgttattgatgacaattaagccattaaaacctataattaattatctttcaattcgagtaaatttaaaacggtgtaaaattaaaatatgatcgtattcttaaatgaataaaactcacttaataatagtaatacttgaatcacatctacgaacatagattcttttcatccagtctaaccatgtttgaatatatagagtttgattatggttatgtctttgtccacattttggtttgtaaataaatgtgcaacggaggtatggtactgttgctctatcaaattcaagtttgaattaaaagaaaaaaaaaaagacgatattttgtgcgctttgtttggtaggtaaaacgagagaacaaacgcattccaaatcatgcggattttgatcggcaacacacaccacaaaaaaccgtacacgatgcacgtgccatttgccgggggtttctaacaaggtaattgggcaggcacgtgatcccccagctacccacctctcgcttcccttctcaaactccttttccatgtatatatacaaccccttttctcagaccattatattctaacatttttgctttgctattgtaacgcaacaaaaactgctcattccatccttgttcctccccattttgatcttctctcgacccttctccgagat

SEQ ID NO: 12 - DNA, 58 bp, Arabidopsis thaliana
  source 1..58: mol_type = other DNA
tacatcacaatcacacaaaactaacaaaagatcaaaagcaagttcttcactgttgata